European Patent Specification EP 3 548 515 B1, published January 21, 2026. Title: RADIOLABELED ANTI-PD-L1 ANTIBODIES FOR IMMUNO-PET IMAGING. Applicant: Regeneron Pharmaceuticals, Inc. Kelly, Marcus Ma, Dangshe Olson, William Thurston, Gavin. Application TBD. The sequence listing filed with the application follows.

SEQUENCE LISTING (344 sequences)

SEQ ID NO: 1 - DNA, 363 bp, Artificial Sequence
  synthetic
gaggtgcagctggtggagtctgggggaggcttggtccagcctggggggtccctgagactctcctgtgcagcctctggattcacctttagtaggttttggatgagctgggtccgccaggctccagggaaggggctggagtgggtggccaacataaaccaagatggaactgagaaatactatgtggactctgtgaagggccgattcaccatctccagagacaacgccaagaactcactgtatctgcaaatgaacagcctgagagccggggacacggctgtgtattactgtgcgaatacgtattacgatttttggagtggtcactttgactactggggccagggaaccctggtcaccgtctcctca

SEQ ID NO: 2 - protein, 121 aa, Artificial Sequence
  synthetic
EVQLVESGGGLVQPGGSLRLSCAASGFTFSRFWMSWVRQAPGKGLEWVANINQDGTEKYYVDSVKGRFTISRDNAKNSLYLQMNSLRAGDTAVYYCANTYYDFWSGHFDYWGQGTLVTVSS

SEQ ID NO: 3 - DNA, 24 bp, Artificial Sequence
  synthetic
ggattcacctttagtaggttttgg

SEQ ID NO: 4 - protein, 8 aa, Artificial Sequence
  synthetic
GFTFSRFW

SEQ ID NO: 5 - DNA, 24 bp, Artificial Sequence
  synthetic
ataaaccaagatggaactgagaaa

SEQ ID NO: 6 - protein, 8 aa, Artificial Sequence
  synthetic
INQDGTEK

SEQ ID NO: 7 - DNA, 42 bp, Artificial Sequence
  synthetic
gcgaatacgtattacgatttttggagtggtcactttgactac

SEQ ID NO: 8 - protein, 14 aa, Artificial Sequence
  synthetic
ANTYYDFWSGHFDY

SEQ ID NO: 9 - DNA, 321 bp, Artificial Sequence
  synthetic
gacatccagatgacccagtctccttccaccctgtctgcatctgtaggagacagagtcaccatcacttgtcgggccagtcagagtattagtaattggttggcctggtatcagcagaaaccagggaaagcccctaagctcctgatctataaggcgtctagtttagaaagtggggtcccatcaaggttcagcggcagtggatctgggacagaattcactctcaccatcagcagcctgcagcctgatgattttgcaacttattactgccaacagtatcatagttattcgtacacttttggccaggggaccaagctggagatcaaa

SEQ ID NO: 10 - protein, 107 aa, Artificial Sequence
  synthetic
DIQMTQSPSTLSASVGDRVTITCRASQSISNWLAWYQQKPGKAPKLLIYKASSLESGVPSRFSGSGSGTEFTLTISSLQPDDFATYYCQQYHSYSYTFGQGTKLEIK

SEQ ID NO: 11 - DNA, 18 bp, Artificial Sequence
  synthetic
cagagtattagtaattgg

SEQ ID NO: 12 - protein, 6 aa, Artificial Sequence
  synthetic
QSISNW

SEQ ID NO: 13 - DNA, 9 bp, Artificial Sequence
  synthetic
aaggcgtct

SEQ ID NO: 14 - protein, 3 aa, Artificial Sequence
  synthetic
KAS

SEQ ID NO: 15 - DNA, 27 bp, Artificial Sequence
  synthetic
caacagtatcatagttattcgtacact

SEQ ID NO: 16 - protein, 9 aa, Artificial Sequence
  synthetic
QQYHSYSYT

SEQ ID NO: 17 - DNA, 363 bp, Artificial Sequence
  synthetic
caggagcacctggtggagtctgggggaggcgtggtccagcctgggaggtccctgagactctcctgtgaagcgtctggattcaccttcagtaactttggcatgcactgggtccgccaggctccaggcaaggggctggagtgggtggcagctttatggtctgatggaagtaataaatactatgcagactccgtgaagggtcgagtcaccatctccagagacaattccaagaacacactgtatctgcaaatgaacagcctgagagccgaggacacggctgtctattactgtgcgagagggagaggagcccccggtattccgatttttgggtactggggccagggaaccctggtcaccgtctcctca

SEQ ID NO: 18 - protein, 121 aa, Artificial Sequence
  synthetic
QEHLVESGGGVVQPGRSLRLSCEASGFTFSNFGMHWVRQAPGKGLEWVAALWSDGSNKYYADSVKGRVTISRDNSKNTLYLQMNSLRAEDTAVYYCARGRGAPGIPIFGYWGQGTLVTVSS

SEQ ID NO: 19 - DNA, 24 bp, Artificial Sequence
  synthetic
ggattcaccttcagtaactttggc

SEQ ID NO: 20 - protein, 8 aa, Artificial Sequence
  synthetic
GFTFSNFG

SEQ ID NO: 21 - DNA, 24 bp, Artificial Sequence
  synthetic
ttatggtctgatggaagtaataaa

SEQ ID NO: 22 - protein, 8 aa, Artificial Sequence
  synthetic
LWSDGSNK

SEQ ID NO: 23 - DNA, 42 bp, Artificial Sequence
  synthetic
gcgagagggagaggagcccccggtattccgatttttgggtac

SEQ ID NO: 24 - protein, 14 aa, Artificial Sequence
  synthetic
ARGRGAPGIPIFGY

SEQ ID NO: 25 - DNA, 321 bp, Artificial Sequence
  synthetic
gacatccagatgacccagtctccatcctccctgtctgcatctgttggagacagagtcaccatcacttgccgggcaagtcagggcattagaaatgatttaggctggtatcagcagaaaccagggaaagcccctaagcgcctgatctatactgcatccagtttgcaaagtggggtcccatcaagattcagcggcagtggatctgggacagaattcactctcacaatcagcagcctacagcctgaagattttgcaacttattactgtctacaacataatagttaccctctcacattcggcggagggaccaaggtggcgatcaaa

SEQ ID NO: 26 - protein, 107 aa, Artificial Sequence
  synthetic
DIQMTQSPSSLSASVGDRVTITCRASQGIRNDLGWYQQKPGKAPKRLIYTASSLQSGVPSRFSGSGSGTEFTLTISSLQPEDFATYYCLQHNSYPLTFGGGTKVAIK

SEQ ID NO: 27 - DNA, 18 bp, Artificial Sequence
  synthetic
cagggcattagaaatgat

SEQ ID NO: 28 - protein, 6 aa, Artificial Sequence
  synthetic
QGIRND

SEQ ID NO: 29 - DNA, 9 bp, Artificial Sequence
  synthetic
actgcatcc

SEQ ID NO: 30 - protein, 3 aa, Artificial Sequence
  synthetic
TAS

SEQ ID NO: 31 - DNA, 27 bp, Artificial Sequence
  synthetic
ctacaacataatagttaccctctcaca

SEQ ID NO: 32 - protein, 9 aa, Artificial Sequence
  synthetic
LQHNSYPLT

SEQ ID NO: 33 - DNA, 390 bp, Artificial Sequence
  synthetic
gaggtgcagctggtggagtctgggggaggcttggtaaagcctggggggtcccttagactctcctgtgcagcctctggattcactttcagtaacgcctggatgagctgggtccgccaggctccagggaaggggctggagtgggttggccgtattaaaaggaaaactgatggtgggacaacagactacgctgcacccgtgaaaggcagattcaccatctcaagagatgattcaaaaaatacgctgcatctgcaaatgaacagcctgaaaaccgaggacacagccgtgtattactgtaccacagatgatattgtagttgtaccagctgttatgagggaatactacttcggtatggacgtctggggccaagggaccacggtcaccgtctcctca

SEQ ID NO: 34 - protein, 130 aa, Artificial Sequence
  synthetic
EVQLVESGGGLVKPGGSLRLSCAASGFTFSNAWMSWVRQAPGKGLEWVGRIKRKTDGGTTDYAAPVKGRFTISRDDSKNTLHLQMNSLKTEDTAVYYCTTDDIVVVPAVMREYYFGMDVWGQGTTVTVSS

SEQ ID NO: 35 - DNA, 24 bp, Artificial Sequence
  synthetic
ggattcactttcagtaacgcctgg

SEQ ID NO: 36 - protein, 8 aa, Artificial Sequence
  synthetic
GFTFSNAW

SEQ ID NO: 37 - DNA, 30 bp, Artificial Sequence
  synthetic
attaaaaggaaaactgatggtgggacaaca

SEQ ID NO: 38 - protein, 10 aa, Artificial Sequence
  synthetic
IKRKTDGGTT

SEQ ID NO: 39 - DNA, 63 bp, Artificial Sequence
  synthetic
accacagatgatattgtagttgtaccagctgttatgagggaatactacttcggtatggacgtc

SEQ ID NO: 40 - protein, 21 aa, Artificial Sequence
  synthetic
TTDDIVVVPAVMREYYFGMDV

SEQ ID NO: 41 - DNA, 321 bp, Artificial Sequence
  synthetic
gacatccagatgacccagtctccatcctccctgtctgcatctgtaggagacagagtcaccatcacttgccggacaagtcagggcattagaaatgatttaggctggtatcagcagaaaccagggaaagcccctaagcgcctgatctatgctgcatccagtttgcaaagtggggtcccatcaaggttcagcggcagtggatctgggacagaattcactctcacaatcagcagcctgcagcctgaagattttgcaacttattactgtctacagcataataattacccgtacacttttggccaggggaccaagctggagatcaaa

SEQ ID NO: 42 - protein, 107 aa, Artificial Sequence
  synthetic
DIQMTQSPSSLSASVGDRVTITCRTSQGIRNDLGWYQQKPGKAPKRLIYAASSLQSGVPSRFSGSGSGTEFTLTISSLQPEDFATYYCLQHNNYPYTFGQGTKLEIK

SEQ ID NO: 43 - DNA, 18 bp, Artificial Sequence
  synthetic
cagggcattagaaatgat

SEQ ID NO: 44 - protein, 6 aa, Artificial Sequence
  synthetic
QGIRND

SEQ ID NO: 45 - DNA, 9 bp, Artificial Sequence
  synthetic
gctgcatcc

SEQ ID NO: 46 - protein, 3 aa, Artificial Sequence
  synthetic
AAS

SEQ ID NO: 47 - DNA, 27 bp, Artificial Sequence
  synthetic
ctacagcataataattacccgtacact

SEQ ID NO: 48 - protein, 9 aa, Artificial Sequence
  synthetic
LQHNNYPYT

SEQ ID NO: 49 - DNA, 363 bp, Artificial Sequence
  synthetic
caggtgcaattggtgcagtctggggcggaggtgaagaagcctggggcctcagtgcaggtctcctgcaaggcttctggatactccttcaccggctactatatacactgggtgcgacaggcccctggacaaggacttgagtggatgggatggatcaaccctaacagtggcaccaaaaagtatgcacacaagtttcagggcagggtcaccatgaccagggacacgtccatcgacacagcctacatgattttgagcagtctgatatccgacgacacggccgtgtattactgtgcgagagatgaggactggaactttgggagctggttcgactcctggggccagggaaccctggtcaccgtctcctca

SEQ ID NO: 50 - protein, 121 aa, Artificial Sequence
  synthetic
QVQLVQSGAEVKKPGASVQVSCKASGYSFTGYYIHWVRQAPGQGLEWMGWINPNSGTKKYAHKFQGRVTMTRDTSIDTAYMILSSLISDDTAVYYCARDEDWNFGSWFDSWGQGTLVTVSS

SEQ ID NO: 51 - DNA, 24 bp, Artificial Sequence
  synthetic
ggatactccttcaccggctactat

SEQ ID NO: 52 - protein, 8 aa, Artificial Sequence
  synthetic
GYSFTGYY

SEQ ID NO: 53 - DNA, 24 bp, Artificial Sequence
  synthetic
atcaaccctaacagtggcaccaaa

SEQ ID NO: 54 - protein, 8 aa, Artificial Sequence
  synthetic
INPNSGTK

SEQ ID NO: 55 - DNA, 42 bp, Artificial Sequence
  synthetic
gcgagagatgaggactggaactttgggagctggttcgactcc

SEQ ID NO: 56 - protein, 14 aa, Artificial Sequence
  synthetic
ARDEDWNFGSWFDS

SEQ ID NO: 57 - DNA, 336 bp, Artificial Sequence
  synthetic
gatattgtgatgacccagactccactctcctcacctgtcacccttggacagccggcctccatctcctgcaggtctagtcaaaccctcgtacacggtgatggaaacacgtacttgagttggattcagcagaggccaggccagcctccgagactcctcatttataaggtttctaatcagttctctggggtcccagacagattcagtggcagtggggcagggacagatttcacactgaaaatcagcagggtggaagctgaggatgtcgggctttatttctgcatgcaagctacacattttccgatcaccttcggccaagggacacgactggagattaaa

SEQ ID NO: 58 - protein, 112 aa, Artificial Sequence
  synthetic
DIVMTQTPLSSPVTLGQPASISCRSSQTLVHGDGNTYLSWIQQRPGQPPRLLIYKVSNQFSGVPDRFSGSGAGTDFTLKISRVEAEDVGLYFCMQATHFPITFGQGTRLEIK

SEQ ID NO: 59 - DNA, 33 bp, Artificial Sequence
  synthetic
caaaccctcgtacacggtgatggaaacacgtac

SEQ ID NO: 60 - protein, 11 aa, Artificial Sequence
  synthetic
QTLVHGDGNTY

SEQ ID NO: 61 - DNA, 9 bp, Artificial Sequence
  synthetic
aaggtttct

SEQ ID NO: 62 - protein, 3 aa, Artificial Sequence
  synthetic
KVS

SEQ ID NO: 63 - DNA, 27 bp, Artificial Sequence
  synthetic
atgcaagctacacattttccgatcacc

SEQ ID NO: 64 - protein, 9 aa, Artificial Sequence
  synthetic
MQATHFPIT

SEQ ID NO: 65 - DNA, 363 bp, Artificial Sequence
  synthetic
caggtacacctggtgcagtctggggctgaggtgaagaagcctggggcctcagtgaaggtctcctgcaaggcttctggatacaccttcaccggctactatatacattgggtgcgacaggcccctggacacgggcttgagtggatgggatggctcaaccctaatactggtaccacaaagtatatacagaactttcagggcagggtcaccatgaccagggacacgtccagcagcacagcctacatggagctgaccaggctgagatctgacgacacggccgtgtattactgtgcgagagatgaggactggaattatgggagctggttcgacacctggggccagggaaccctggtcacagtctcctca

SEQ ID NO: 66 - protein, 121 aa, Artificial Sequence
  synthetic
QVHLVQSGAEVKKPGASVKVSCKASGYTFTGYYIHWVRQAPGHGLEWMGWLNPNTGTTKYIQNFQGRVTMTRDTSSSTAYMELTRLRSDDTAVYYCARDEDWNYGSWFDTWGQGTLVTVSS

SEQ ID NO: 67 - DNA, 24 bp, Artificial Sequence
  synthetic
ggatacaccttcaccggctactat

SEQ ID NO: 68 - protein, 8 aa, Artificial Sequence
  synthetic
GYTFTGYY

SEQ ID NO: 69 - DNA, 24 bp, Artificial Sequence
  synthetic
ctcaaccctaatactggtaccaca

SEQ ID NO: 70 - protein, 8 aa, Artificial Sequence
  synthetic
LNPNTGTT

SEQ ID NO: 71 - DNA, 42 bp, Artificial Sequence
  synthetic
gcgagagatgaggactggaattatgggagctggttcgacacc

SEQ ID NO: 72 - protein, 14 aa, Artificial Sequence
  synthetic
ARDEDWNYGSWFDT

SEQ ID NO: 73 - DNA, 336 bp, Artificial Sequence
  synthetic
gatattgtaatgacccagactccactctcctcacctgtcacccttggacagccggcctccatctcctgcaggtctagtccaagcctcgtacacagtgatggaaacacctacttgagttggcttcagcagaggccaggccagcctccaagactcctaatttataagatttctaaccgattctctggggtcccagacagattcagtggcagtggggcagggacagatttcacgctgaaaatcagcagggtggaagctgaggatgtcggggtttattactgcatgcaagctacacattttccgatcaccttcggccaagggacacgactggagattaga

SEQ ID NO: 74 - protein, 112 aa, Artificial Sequence
  synthetic
DIVMTQTPLSSPVTLGQPASISCRSSPSLVHSDGNTYLSWLQQRPGQPPRLLIYKISNRFSGVPDRFSGSGAGTDFTLKISRVEAEDVGVYYCMQATHFPITFGQGTRLEIR

SEQ ID NO: 75 - DNA, 33 bp, Artificial Sequence
  synthetic
ccaagcctcgtacacagtgatggaaacacctac

SEQ ID NO: 76 - protein, 11 aa, Artificial Sequence
  synthetic
PSLVHSDGNTY

SEQ ID NO: 77 - DNA, 9 bp, Artificial Sequence
  synthetic
aagatttct

SEQ ID NO: 78 - protein, 3 aa, Artificial Sequence
  synthetic
KIS

SEQ ID NO: 79 - DNA, 27 bp, Artificial Sequence
  synthetic
atgcaagctacacattttccgatcacc

SEQ ID NO: 80 - protein, 9 aa, Artificial Sequence
  synthetic
MQATHFPIT

SEQ ID NO: 81 - DNA, 360 bp, Artificial Sequence
  synthetic
gaggtgcagctggtggaatctgggggaggtgtggtgcggcctggggggtccctgagactctcctgtgcagcctctggattcacttttgatgattatggcatgacctgggtccgccaagctccagggaggggcctggaatgggtctctggtattcattggcatggtaaacgcacaggttatgcagactctgtgaagggccgattcaccatatccagagacaacgccaagaaatccctgtatctgcaaatgaacagtctgaaaggcgaggacacggccttgtatcattgtgtgagggggggaatgagtacaggggactggttcgacccctggggccagggaaccctggtcatcgtctcctca

SEQ ID NO: 82 - protein, 120 aa, Artificial Sequence
  synthetic
EVQLVESGGGVVRPGGSLRLSCAASGFTFDDYGMTWVRQAPGRGLEWVSGIHWHGKRTGYADSVKGRFTISRDNAKKSLYLQMNSLKGEDTALYHCVRGGMSTGDWFDPWGQGTLVIVSS

SEQ ID NO: 83 - DNA, 24 bp, Artificial Sequence
  synthetic
ggattcacttttgatgattatggc

SEQ ID NO: 84 - protein, 8 aa, Artificial Sequence
  synthetic
GFTFDDYG

SEQ ID NO: 85 - DNA, 24 bp, Artificial Sequence
  synthetic
attcattggcatggtaaacgcaca

SEQ ID NO: 86 - protein, 8 aa, Artificial Sequence
  synthetic
IHWHGKRT

SEQ ID NO: 87 - DNA, 39 bp, Artificial Sequence
  synthetic
gtgagggggggaatgagtacaggggactggttcgacccc

SEQ ID NO: 88 - protein, 13 aa, Artificial Sequence
  synthetic
VRGGMSTGDWFDP

SEQ ID NO: 89 - DNA, 324 bp, Artificial Sequence
  synthetic
gacatccagatgacccagtctccatcctccctgtctgcatctctaggagacagagtcaccatcacttgccgggcaagtcagagcattaacagttatttaaattggtatcagcagaaaccagggaaagcccctaaactcctgatctatgttgcatccagtttgcaaagtggggtcccatcaaggttcagtggcagtggatctgggacagaattcactctcaccatcagcaatctgcaacctgaagattttgcaacttactactgtcaacagagttacagtacccctccgatcaccttcggccaagggacacgactggagattaaa

SEQ ID NO: 90 - protein, 108 aa, Artificial Sequence
  synthetic
DIQMTQSPSSLSASLGDRVTITCRASQSINSYLNWYQQKPGKAPKLLIYVASSLQSGVPSRFSGSGSGTEFTLTISNLQPEDFATYYCQQSYSTPPITFGQGTRLEIK

SEQ ID NO: 91 - DNA, 18 bp, Artificial Sequence
  synthetic
cagagcattaacagttat

SEQ ID NO: 92 - protein, 6 aa, Artificial Sequence
  synthetic
QSINSY

SEQ ID NO: 93 - DNA, 9 bp, Artificial Sequence
  synthetic
gttgcatcc

SEQ ID NO: 94 - protein, 3 aa, Artificial Sequence
  synthetic
VAS

SEQ ID NO: 95 - DNA, 30 bp, Artificial Sequence
  synthetic
caacagagttacagtacccctccgatcacc

SEQ ID NO: 96 - protein, 10 aa, Artificial Sequence
  synthetic
QQSYSTPPIT

SEQ ID NO: 97 - DNA, 360 bp, Artificial Sequence
  synthetic
gaggtgcagctggtggagtctgggggaggtgtggtacggccgggggggtccctgagactctcctgtgcagcctctggattcacctttgatgattatggcatgacctgggtccgccaagttccagggaaggggctggagtgggtctctggtattcattggagtggtagaagcacaggttatgcagactctgtgaagggccgattcaccatctccagagacaacgccaagaactccctgtatctgcaaatgaacagtctgagagccgaggacacggccttgtattactgtgcgagggggggaatgagtacgggggactggttcgacccctggggccagggaaccctggtcaccgtctcctca

SEQ ID NO: 98 - protein, 120 aa, Artificial Sequence
  synthetic
EVQLVESGGGVVRPGGSLRLSCAASGFTFDDYGMTWVRQVPGKGLEWVSGIHWSGRSTGYADSVKGRFTISRDNAKNSLYLQMNSLRAEDTALYYCARGGMSTGDWFDPWGQGTLVTVSS

SEQ ID NO: 99 - DNA, 24 bp, Artificial Sequence
  synthetic
ggattcacctttgatgattatggc

SEQ ID NO: 100 - protein, 8 aa, Artificial Sequence
  synthetic
GFTFDDYG

SEQ ID NO: 101 - DNA, 24 bp, Artificial Sequence
  synthetic
attcattggagtggtagaagcaca

SEQ ID NO: 102 - protein, 8 aa, Artificial Sequence
  synthetic
IHWSGRST

SEQ ID NO: 103 - DNA, 39 bp, Artificial Sequence
  synthetic
gcgagggggggaatgagtacgggggactggttcgacccc

SEQ ID NO: 104 - protein, 13 aa, Artificial Sequence
  synthetic
ARGGMSTGDWFDP

SEQ ID NO: 105 - DNA, 324 bp, Artificial Sequence
  synthetic
gacatccagatgacccagtctccatcctccctgtctgcatctgtaggagacagagtcaccatcacttgccgggcaagtcagagcattagcagctatttaaattggtatcagcagaaaccagggaaagcccctaagctcctgatctatgttgcatccagtttgcaaagtggggtcccatcaaggttcagtggcagtggatctgggacagatttcactctcaccatcagcagtctgcaacctgaagattttgcaacttactactgtcaacagagttacagtacccctccgatcaccttcggccaagggacacgactggagattaaa

SEQ ID NO: 106 - protein, 108 aa, Artificial Sequence
  synthetic
DIQMTQSPSSLSASVGDRVTITCRASQSISSYLNWYQQKPGKAPKLLIYVASSLQSGVPSRFSGSGSGTDFTLTISSLQPEDFATYYCQQSYSTPPITFGQGTRLEIK

SEQ ID NO: 107 - DNA, 18 bp, Artificial Sequence
  synthetic
cagagcattagcagctat

SEQ ID NO: 108 - protein, 6 aa, Artificial Sequence
  synthetic
QSISSY

SEQ ID NO: 109 - DNA, 9 bp, Artificial Sequence
  synthetic
gttgcatcc

SEQ ID NO: 110 - protein, 3 aa, Artificial Sequence
  synthetic
VAS

SEQ ID NO: 111 - DNA, 30 bp, Artificial Sequence; identical to SEQ ID NO: 95
  synthetic

SEQ ID NO: 112 - protein, 10 aa, Artificial Sequence
  synthetic
QQSYSTPPIT

SEQ ID NO: 113 - DNA, 345 bp, Artificial Sequence
  synthetic
gaggtgcagttggtggagtctggaggaggcttggtccagcctggggggtccctaagactctcctgtgcagcctctgggttcaccgtcggtagtaactacatgaactgggtccgtcaggctccagggaagggactggagtgggtctcagttatttatagtggtggtagtacatactacgcagattccgtgaagggccgattcaccatctccagactcacttccaagaacacactgtatcttcaaatgagcagcctgagacctgaggacacggccgtgtattattgtgcgagagggattaggggtctggacgtctggggccaagggaccacggtcaccgtctcttca

SEQ ID NO: 114 - protein, 115 aa, Artificial Sequence
  synthetic
EVQLVESGGGLVQPGGSLRLSCAASGFTVGSNYMNWVRQAPGKGLEWVSVIYSGGSTYYADSVKGRFTISRLTSKNTLYLQMSSLRPEDTAVYYCARGIRGLDVWGQGTTVTVSS

SEQ ID NO: 115 - DNA, 24 bp, Artificial Sequence
  synthetic
gggttcaccgtcggtagtaactac

SEQ ID NO: 116 - protein, 8 aa, Artificial Sequence
  synthetic
GFTVGSNY

SEQ ID NO: 117 - DNA, 21 bp, Artificial Sequence
  synthetic
atttatagtggtggtagtaca

SEQ ID NO: 118 - protein, 7 aa, Artificial Sequence
  synthetic
IYSGGST

SEQ ID NO: 119 - DNA, 27 bp, Artificial Sequence
  synthetic
gcgagagggattaggggtctggacgtc

SEQ ID NO: 120 - protein, 9 aa, Artificial Sequence
  synthetic
ARGIRGLDV

SEQ ID NO: 121 - DNA, 324 bp, Artificial Sequence
  synthetic
gacatccagatgacccagtctccatcctccctgtctgcatctgtaggagacagagtcaccatcacttgccgggcaagtcagaccattaacatctatttaaattggtatcagcagaaaccagggagagcccctaggctcctgatctatgctgcatccagtttgcaaagtggggtcccatcaaggttcagtggcagtggatctgggacagatttcactctcaccatcagcagtctgcaacctgaagattttgcaacttactactgtcaccagagttacagtacccctccgatcaccttcggccaagggacacgactggagattaaa

SEQ ID NO: 122 - protein, 108 aa, Artificial Sequence
  synthetic
DIQMTQSPSSLSASVGDRVTITCRASQTINIYLNWYQQKPGRAPRLLIYAASSLQSGVPSRFSGSGSGTDFTLTISSLQPEDFATYYCHQSYSTPPITFGQGTRLEIK

SEQ ID NO: 123 - DNA, 18 bp, Artificial Sequence
  synthetic
cagaccattaacatctat

SEQ ID NO: 124 - protein, 6 aa, Artificial Sequence
  synthetic
QTINIY

SEQ ID NO: 125 - DNA, 9 bp, Artificial Sequence
  synthetic
gctgcatcc

SEQ ID NO: 126 - protein, 3 aa, Artificial Sequence
  synthetic
AAS

SEQ ID NO: 127 - DNA, 30 bp, Artificial Sequence
  synthetic
caccagagttacagtacccctccgatcacc

SEQ ID NO: 128 - protein, 10 aa, Artificial Sequence
  synthetic
HQSYSTPPIT

SEQ ID NO: 129 - DNA, 345 bp, Artificial Sequence
  synthetic
gaggaacggttggtggagtctggaggagacttggtccagcctggggggtccctgagactctcctgtgcagcctctggcatcaccgtcggtactaattatatgaactgggtccgccaggctccagggaagggactggagtgggtctcagttatttctagcggtggtaatacacactacgcagactccgtgaagggccgattcattatgtccagacaaacttccaaaaacacgctgtatcttcagatgaatagcctggaaactgaggacacggccgtatattattgtgcgagggggatcagaggtttggacgtctggggccaagggaccatggtcaccgtctcctca

SEQ ID NO: 130 - protein, 115 aa, Artificial Sequence
  synthetic
EERLVESGGDLVQPGGSLRLSCAASGITVGTNYMNWVRQAPGKGLEWVSVISSGGNTHYADSVKGRFIMSRQTSKNTLYLQMNSLETEDTAVYYCARGIRGLDVWGQGTMVTVSS

SEQ ID NO: 131 - DNA, 24 bp, Artificial Sequence
  synthetic
ggcatcaccgtcggtactaattat

SEQ ID NO: 132 - protein, 8 aa, Artificial Sequence
  synthetic
GITVGTNY

SEQ ID NO: 133 - DNA, 21 bp, Artificial Sequence
  synthetic
atttctagcggtggtaataca

SEQ ID NO: 134 - protein, 7 aa, Artificial Sequence
  synthetic
ISSGGNT

SEQ ID NO: 135 - DNA, 27 bp, Artificial Sequence
  synthetic
gcgagggggatcagaggtttggacgtc

SEQ ID NO: 136 - protein, 9 aa, Artificial Sequence
  synthetic
ARGIRGLDV

SEQ ID NO: 137 - DNA, 324 bp, Artificial Sequence
  synthetic
gacatccagatgacccagtctccatcctccctgtctgcatctgtaggagacagagtcaccatcacttgccgggcaagtcagagcatgagcagctatttaaattggtatcagcagaaaccagggagagcccctaagctcctgatctttgctgcatccagtttgcaaagtggggtcccatcaaggttcagtggcagtggatctgggacagatttcactctcaccatcagcagtctgcaacctgaagattttgcaacttactactgtcaacagagttacagtacccctccgatcaccttcggccaagggacacgactggagattaaa

SEQ ID NO: 138 - protein, 108 aa, Artificial Sequence
  synthetic
DIQMTQSPSSLSASVGDRVTITCRASQSMSSYLNWYQQKPGRAPKLLIFAASSLQSGVPSRFSGSGSGTDFTLTISSLQPEDFATYYCQQSYSTPPITFGQGTRLEIK

SEQ ID NO: 139 - DNA, 18 bp, Artificial Sequence
  synthetic
cagagcatgagcagctat

SEQ ID NO: 140 - protein, 6 aa, Artificial Sequence
  synthetic
QSMSSY

SEQ ID NO: 141 - DNA, 9 bp, Artificial Sequence
  synthetic
gctgcatcc

SEQ ID NO: 142 - protein, 3 aa, Artificial Sequence
  synthetic
AAS

SEQ ID NO: 143 - DNA, 30 bp, Artificial Sequence; identical to SEQ ID NO: 95
  synthetic

SEQ ID NO: 144 - protein, 10 aa, Artificial Sequence
  synthetic
QQSYSTPPIT

SEQ ID NO: 145 - DNA, 354 bp, Artificial Sequence
  synthetic
caggtccagctggtgcagtctggggctgaggtgaagatgcctgggtcctcggtgagggtctcctgcaaggcttctggaggcatcttcagcagttctactatcagttgggtgcgacaggcccctggacaagggcttgaatggatgggagagatcatccctgtctttggtacagtaaactacgcacagaagttccaggacagagtcatatttaccgcggacgaatctacgactacagcctacatggagctgagcagcctgaaatctggggacacggccgtatatttctgtgcgcgaaattggggattaggctctttttatatctggggccaagggacaatggtcaccgtctcttca

SEQ ID NO: 146 - protein, 118 aa, Artificial Sequence
  synthetic
QVQLVQSGAEVKMPGSSVRVSCKASGGIFSSSTISWVRQAPGQGLEWMGEIIPVFGTVNYAQKFQDRVIFTADESTTTAYMELSSLKSGDTAVYFCARNWGLGSFYIWGQGTMVTVSS

SEQ ID NO: 147 - DNA, 24 bp, Artificial Sequence
  synthetic
ggaggcatcttcagcagttctact

SEQ ID NO: 148 - protein, 8 aa, Artificial Sequence
  synthetic
GGIFSSST

SEQ ID NO: 149 - DNA, 24 bp, Artificial Sequence
  synthetic
atcatccctgtctttggtacagta

SEQ ID NO: 150 - protein, 8 aa, Artificial Sequence
  synthetic
IIPVFGTV

SEQ ID NO: 151 - DNA, 33 bp, Artificial Sequence
  synthetic
gcgcgaaattggggattaggctctttttatatc

SEQ ID NO: 152 - protein, 11 aa, Artificial Sequence
  synthetic
ARNWGLGSFYI

SEQ ID NO: 153 - DNA, 324 bp, Artificial Sequence
  synthetic
gaaattgtgttgacgcagtctccaggcaccctgtctttgtctccaggggaaagagccaccctctcctgcagggccagtcagagttttaacttcaactacttagcctggtaccagcagaaacctggccaggctcccagactcctcatctatggtgcatccagcagggccactggcatcccagacaggttcagtggcagtgggtctgggacagacttcactctcaccatcaacaggctggagcctgaagattttggagtgttttattgtcagcagtatgaaagcgcaccttggacgttcggccaagggaccaaggtggaaatcaaa

SEQ ID NO: 154 - protein, 108 aa, Artificial Sequence
  synthetic
EIVLTQSPGTLSLSPGERATLSCRASQSFNFNYLAWYQQKPGQAPRLLIYGASSRATGIPDRFSGSGSGTDFTLTINRLEPEDFGVFYCQQYESAPWTFGQGTKVEIK

SEQ ID NO: 155 - DNA, 21 bp, Artificial Sequence
  synthetic
cagagttttaacttcaactac

SEQ ID NO: 156 - protein, 7 aa, Artificial Sequence
  synthetic
QSFNFNY

SEQ ID NO: 157 - DNA, 9 bp, Artificial Sequence
  synthetic
ggtgcatcc

SEQ ID NO: 158 - protein, 3 aa, Artificial Sequence
  synthetic
GAS

SEQ ID NO: 159 - DNA, 27 bp, Artificial Sequence
  synthetic
cagcagtatgaaagcgcaccttggacg

SEQ ID NO: 160 - protein, 9 aa, Artificial Sequence
  synthetic
QQYESAPWT

SEQ ID NO: 161 - DNA, 345 bp, Artificial Sequence
  synthetic
gaggtgcagcttgtagagtctgggggagacttggtacatcctggcaggtccctgagactctcctgtgcagcctctggtttcccctttgatgagtatgccatgcactgggtccggcaagttccagggaagggcctggagtgggtctcaggtattagttggagtaataataacataggctatgcggactctgtgaagggccgattcaccatctccagagacaacgccaaaaactccctgtatctacaaatgaacagtctgagacctgaggacacggccttttattactgtgcaaaatctggaatctttgactcctggggccagggaaccctggtcaccgtctcctca

SEQ ID NO: 162 - protein, 115 aa, Artificial Sequence
  synthetic
EVQLVESGGDLVHPGRSLRLSCAASGFPFDEYAMHWVRQVPGKGLEWVSGISWSNNNIGYADSVKGRFTISRDNAKNSLYLQMNSLRPEDTAFYYCAKSGIFDSWGQGTLVTVSS

SEQ ID NO: 163 - DNA, 24 bp, Artificial Sequence
  synthetic
ggtttcccctttgatgagtatgcc

SEQ ID NO: 164 - protein, 8 aa, Artificial Sequence
  synthetic
GFPFDEYA

SEQ ID NO: 165 - DNA, 24 bp, Artificial Sequence
  synthetic
attagttggagtaataataacata

SEQ ID NO: 166 - protein, 8 aa, Artificial Sequence
  synthetic
ISWSNNNI

SEQ ID NO: 167 - DNA, 24 bp, Artificial Sequence
  synthetic
gcaaaatctggaatctttgactcc

SEQ ID NO: 168 - protein, 8 aa, Artificial Sequence
  synthetic
AKSGIFDS

SEQ ID NO: 169 - DNA, 315 bp, Artificial Sequence
  synthetic
gacatccagatgacccagtctccatcctccctgtctgcatctgtaggagacagagtcaccatcacttgccgggcaagtcagagcattagcagctatttaaattggtatcagcagaaaccagggaagctcctgatctatgctgcatccagtttgcaaagtggggtcccatcacggttcagtggcggtggatctgggacagatttcactctcaccatcagcagtctgcgacctgaagattttgcaacttactactgtcaacagagttactgtacccctccgatcaccttcggccaagggacacgactggagattaaa

SEQ ID NO: 170 - protein, 105 aa, Artificial Sequence
  synthetic
DIQMTQSPSSLSASVGDRVTITCRASQSISSYLNWYQQKPGKLLIYAASSLQSGVPSRFSGGGSGTDFTLTISSLRPEDFATYYCQQSYCTPPITFGQGTRLEIK

SEQ ID NO: 171 - DNA, 18 bp, Artificial Sequence
  synthetic
cagagcattagcagctat

SEQ ID NO: 172 - protein, 6 aa, Artificial Sequence
  synthetic
QSISSY

SEQ ID NO: 173 - DNA, 9 bp, Artificial Sequence
  synthetic
gctgcatcc

SEQ ID NO: 174 - protein, 3 aa, Artificial Sequence
  synthetic
AAS

SEQ ID NO: 175 - DNA, 30 bp, Artificial Sequence
  synthetic
caacagagttactgtacccctccgatcacc

SEQ ID NO: 176 - protein, 10 aa, Artificial Sequence
  synthetic
QQSYCTPPIT

SEQ ID NO: 177 - DNA, 354 bp, Artificial Sequence
  synthetic
gaggtgcagctggtggagtccgggggaggcgtggtccagcctgggaggtccctgagactctcctgtgcagcctctggattcaccttcagtagttatggcatgcactgggtccgccaggctccaggcaagggactggagtgggtgacacttatatcatatgagggaaggaataaatactatgcagactccgtgaagggccgattcaccatttccagagacaattccaagaacacgctgtatctgcaaatgaacagcctgagagctgaggacacggctgtatattactgtgcgaaagataggaccctttacggtatggacgtctggggccaaggaaccacggtcaccgtctcctca

SEQ ID NO: 178 - protein, 118 aa, Artificial Sequence
  synthetic
EVQLVESGGGVVQPGRSLRLSCAASGFTFSSYGMHWVRQAPGKGLEWVTLISYEGRNKYYADSVKGRFTISRDNSKNTLYLQMNSLRAEDTAVYYCAKDRTLYGMDVWGQGTTVTVSS

SEQ ID NO: 179 - DNA, 24 bp, Artificial Sequence
  synthetic
ggattcaccttcagtagttatggc

SEQ ID NO: 180 - protein, 8 aa, Artificial Sequence
  synthetic
GFTFSSYG

SEQ ID NO: 181 - DNA, 24 bp, Artificial Sequence
  synthetic
atatcatatgagggaaggaataaa

SEQ ID NO: 182 - protein, 8 aa, Artificial Sequence
  synthetic
ISYEGRNK

SEQ ID NO: 183 - DNA, 33 bp, Artificial Sequence
  synthetic
gcgaaagataggaccctttacggtatggacgtc

SEQ ID NO: 184 - protein, 11 aa, Artificial Sequence
  synthetic
AKDRTLYGMDV

SEQ ID NO: 185 - DNA, 363 bp, Artificial Sequence
  synthetic
caggtcaccttgagggagtctggtcctgcgctggtgaaaaccacacagaccctcacactgacctgcaccttctctgggttctcactcagcactaatagaatgtgtgtgacctggatccgtcagcccccagggaaggccctggagtggcttgcgcgcattgattgggatggtgttaaatactacaacacatctctgaagaccaggctcaccatctccaaggacacctccaaaaaccaggtggtccttacaatgaccaacatggaccctgtggacacagccactttttactgtgcacggtcgacttcgttgactttttactactttgactactggggccagggaaccctggtcaccgtctcctca

SEQ ID NO: 186 - protein, 121 aa, Artificial Sequence
  synthetic
QVTLRESGPALVKTTQTLTLTCTFSGFSLSTNRMCVTWIRQPPGKALEWLARIDWDGVKYYNTSLKTRLTISKDTSKNQVVLTMTNMDPVDTATFYCARSTSLTFYYFDYWGQGTLVTVSS

SEQ ID NO: 187 - DNA, 30 bp, Artificial Sequence
  synthetic
gggttctcactcagcactaatagaatgtgt

SEQ ID NO: 188 - protein, 10 aa, Artificial Sequence
  synthetic
GFSLSTNRMC

SEQ ID NO: 189 - DNA, 21 bp, Artificial Sequence
  synthetic
attgattgggatggtgttaaa

SEQ ID NO: 190 - protein, 7 aa, Artificial Sequence
  synthetic
IDWDGVK

SEQ ID NO: 191 - DNA, 39 bp, Artificial Sequence
  synthetic
gcacggtcgacttcgttgactttttactactttgactac

SEQ ID NO: 192 - protein, 13 aa, Artificial Sequence
  synthetic
ARSTSLTFYYFDY

SEQ ID NO: 193 - DNA, 324 bp, Artificial Sequence
  synthetic
gacatccagatgacccagtctccatcctccctgtctgcatctgtaggagacagagtcaccatcacttgccgggcaagtcagagcattagcagctatttaaattggtatcagcagaaaccagggaaagcccctaagctcctgatctatgctgcatccagtttgcaaagtggggtcccatcaaggttcagtggcagtggatctgggacagatttcactctcaccatcagcagtctgcaacctgaagattttgcaacttactactgtcaacagagttacagtacccctccgatcaccttcggccaagggacacgactggagattaaa

SEQ ID NO: 194 - protein, 108 aa, Artificial Sequence
  synthetic
DIQMTQSPSSLSASVGDRVTITCRASQSISSYLNWYQQKPGKAPKLLIYAASSLQSGVPSRFSGSGSGTDFTLTISSLQPEDFATYYCQQSYSTPPITFGQGTRLEIK

SEQ ID NO: 195 - DNA, 18 bp, Artificial Sequence
  synthetic
cagagcattagcagctat

SEQ ID NO: 196 - protein, 6 aa, Artificial Sequence
  synthetic
QSISSY

SEQ ID NO: 197 - DNA, 9 bp, Artificial Sequence
  synthetic
gctgcatcc

SEQ ID NO: 198 - protein, 3 aa, Artificial Sequence
  synthetic
AAS

SEQ ID NO: 199 - DNA, 30 bp, Artificial Sequence; identical to SEQ ID NO: 95
  synthetic

SEQ ID NO: 200 - protein, 10 aa, Artificial Sequence
  synthetic
QQSYSTPPIT

SEQ ID NO: 201 - DNA, 345 bp, Artificial Sequence
  synthetic
gaggtgcagctggtggagtctggaggaggcttggtccagccgggggggtccctgagactctcctgtgcagcctctgagttcaccgtcggtaccaaccacatgaactgggtccgccaggctccagggaagggactggagtgggtctcagttatttatagcggtggtaacacattctacgcagactccgtgaagggccgattcaccatctccagacacacttccaagaacacgctgtatcttcaaatgaacagcctgacagcagaggacacggccgtatattactgtgcgcgaggattggggggtatggacgtctggggccaagggaccacggtcaccgtctcctca

SEQ ID NO: 202 - protein, 115 aa, Artificial Sequence
  synthetic
EVQLVESGGGLVQPGGSLRLSCAASEFTVGTNHMNWVRQAPGKGLEWVSVIYSGGNTFYADSVKGRFTISRHTSKNTLYLQMNSLTAEDTAVYYCARGLGGMDVWGQGTTVTVSS

SEQ ID NO: 203 - DNA, 24 bp, Artificial Sequence
  synthetic
gagttcaccgtcggtaccaaccac

SEQ ID NO: 204 - protein, 8 aa, Artificial Sequence
  synthetic
EFTVGTNH

SEQ ID NO: 205 - DNA, 21 bp, Artificial Sequence
  synthetic
atttatagcggtggtaacaca

SEQ ID NO: 206 - protein, 7 aa, Artificial Sequence
  synthetic
IYSGGNT

SEQ ID NO: 207 - DNA, 27 bp, Artificial Sequence
  synthetic
gcgcgaggattggggggtatggacgtc

SEQ ID NO: 208 - protein, 9 aa, Artificial Sequence
  synthetic
ARGLGGMDV

SEQ ID NO: 209 - DNA, 321 bp, Artificial Sequence
  synthetic
gacatccagatgacccagtctccatcctccctgtctgcatctgtaggagacagagtcaccatcacttgccgggcgagtcaggtcattagcaattatttagcctggtatcagcagaaaccagggaaagttcctaggctcctgatctatgctgcatccactttgcaatcaggggtcccatctcgtttcagtggcagtggatctgggacagatttcactctcaccatcagcagcctgcagcctgaagatgttgcaacttattactgtcaaaagtataacagtgcccctcggacgttcggccaagggaccaaggtggaaatcaaa

SEQ ID NO: 210 - protein, 107 aa, Artificial Sequence
  synthetic
DIQMTQSPSSLSASVGDRVTITCRASQVISNYLAWYQQKPGKVPRLLIYAASTLQSGVPSRFSGSGSGTDFTLTISSLQPEDVATYYCQKYNSAPRTFGQGTKVEIK

SEQ ID NO: 211 - DNA, 18 bp, Artificial Sequence
  synthetic
caggtcattagcaattat

SEQ ID NO: 212 - protein, 6 aa, Artificial Sequence
  synthetic
QVISNY

SEQ ID NO: 213 - DNA, 9 bp, Artificial Sequence
  synthetic
gctgcatcc

SEQ ID NO: 214 - protein, 3 aa, Artificial Sequence
  synthetic
AAS

SEQ ID NO: 215 - DNA, 27 bp, Artificial Sequence
  synthetic
caaaagtataacagtgcccctcggacg

SEQ ID NO: 216 - protein, 9 aa, Artificial Sequence
  synthetic
QKYNSAPRT

SEQ ID NO: 217 - DNA, 360 bp, Artificial Sequence
  synthetic
gaggtgcagctggtggagtctgggggaggcttggtccagcggggggagtccctgagactttactgtgcagcctctggattcacctttagtaaatattggatgaactgggtccgccaggctccagggaaggggctggagtgggtggccaacataaagggagatggaagtgagaaatactatgtggactctgtgaagggccggttcaccatctccagagacaacgccaagaactcactatatctacaaatgaacagcctgagagccgaggacacggctgtttattactgtgcgagagattattggggatcaggctactactttgacttctggggccagggaaccctggtcaccgtctcctca

SEQ ID NO: 218 - protein, 120 aa, Artificial Sequence
  synthetic
EVQLVESGGGLVQRGESLRLYCAASGFTFSKYWMNWVRQAPGKGLEWVANIKGDGSEKYYVDSVKGRFTISRDNAKNSLYLQMNSLRAEDTAVYYCARDYWGSGYYFDFWGQGTLVTVSS

SEQ ID NO: 219 - DNA, 24 bp, Artificial Sequence
  synthetic
ggattcacctttagtaaatattgg

SEQ ID NO: 220 - protein, 8 aa, Artificial Sequence
  synthetic
GFTFSKYW

SEQ ID NO: 221 - DNA, 24 bp, Artificial Sequence
  synthetic
ataaagggagatggaagtgagaaa

SEQ ID NO: 222 - protein, 8 aa, Artificial Sequence
  synthetic
IKGDGSEK

SEQ ID NO: 223 - DNA, 39 bp, Artificial Sequence
  synthetic
gcgagagattattggggatcaggctactactttgacttc

SEQ ID NO: 224 - protein, 13 aa, Artificial Sequence
  synthetic
ARDYWGSGYYFDF

SEQ ID NO: 225 - DNA, 321 bp, Artificial Sequence
  synthetic
gacatccagatgacccagtctccatcctccctgtctgcatctgtaggagacagagtcaccatcacttgccgggcaagtcagaacattaacaactatttaaattggtatcagcagaaaccagggaaagcccctaaactcctgatctatgctgcatccagtttccaaaatgcggtcccatcaaggttcagtggcagtggatctgggacagatttcactctcaccatcagcagtctgcaacctgaagattttgcaacttactactgtcaacagagttacaataccccgctcactttcggcggggggaccaaggtggagatcaaa

SEQ ID NO: 226 - protein, 107 aa, Artificial Sequence
  synthetic
DIQMTQSPSSLSASVGDRVTITCRASQNINNYLNWYQQKPGKAPKLLIYAASSFQNAVPSRFSGSGSGTDFTLTISSLQPEDFATYYCQQSYNTPLTFGGGTKVEIK

SEQ ID NO: 227 - DNA, 18 bp, Artificial Sequence
  synthetic
cagaacattaacaactat

SEQ ID NO: 228 - protein, 6 aa, Artificial Sequence
  synthetic
QNINNY

SEQ ID NO: 229 - DNA, 9 bp, Artificial Sequence
  synthetic
gctgcatcc

SEQ ID NO: 230 - protein, 3 aa, Artificial Sequence
  synthetic
AAS

SEQ ID NO: 231 - DNA, 27 bp, Artificial Sequence
  synthetic
caacagagttacaataccccgctcact

SEQ ID NO: 232 - protein, 9 aa, Artificial Sequence
  synthetic
QQSYNTPLT

SEQ ID NO: 233 - DNA, 390 bp, Artificial Sequence
  synthetic
gaggtgcagctggtggagtctgggggaggcttggtccagtctggggggtccctgagactctcctgtgcagcctctggattcacctttagtagctattggatgagctgggtccgccaggctccagggaaggggctggagtgggtggccaacataaagcaagatggaagtgagaaatactatgtggactctgtgaagggccgattcaccatctccagagacaacgccaagaactcactgtatctgcaaatgaacagcctgagagccgatgacacggctgtgtattactgtgcgagagatgatattgtagtagtaccagctcctatgggatattactactactacttcggtatggacgtctggggccaagggaccacggtcaccgtctcctca

SEQ ID NO: 234 - protein, 130 aa, Artificial Sequence
  synthetic
EVQLVESGGGLVQSGGSLRLSCAASGFTFSSYWMSWVRQAPGKGLEWVANIKQDGSEKYYVDSVKGRFTISRDNAKNSLYLQMNSLRADDTAVYYCARDDIVVVPAPMGYYYYYFGMDVWGQGTTVTVSS

SEQ ID NO: 235 - DNA, 24 bp, Artificial Sequence
  synthetic
ggattcacctttagtagctattgg

SEQ ID NO: 236 - protein, 8 aa, Artificial Sequence
  synthetic
GFTFSSYW

SEQ ID NO: 237 - DNA, 24 bp, Artificial Sequence
  synthetic
ataaagcaagatggaagtgagaaa

SEQ ID NO: 238 - protein, 8 aa, Artificial Sequence
  synthetic
IKQDGSEK

SEQ ID NO: 239 - DNA, 69 bp, Artificial Sequence
  synthetic
gcgagagatgatattgtagtagtaccagctcctatgggatattactactactacttcggtatggacgtc

SEQ ID NO: 240 - protein, 23 aa, Artificial Sequence
  synthetic
ARDDIVVVPAPMGYYYYYFGMDV

SEQ ID NO: 241 - DNA, 321 bp, Artificial Sequence
  synthetic
gacatccagatgacccagtctccatcctccctgtctgcatctgtaggagacagagtcaccatcacttgccgggcaagtcagggcattagaaatgatttaggctggtatcagcagaaaccagggaaagcccctaagcgcctgatctatgctgcatccagtttgcaaagtggggtcccatcaaggttcagcggcagtggatctgggacagaattcactctcacaatcagcagcctgcagcctgaagattttgcaacttattactgtctacagcataatagttacccgtacacttttggccaggggaccaagctggagatcaaa

SEQ ID NO: 242 - protein, 107 aa, Artificial Sequence
  synthetic
DIQMTQSPSSLSASVGDRVTITCRASQGIRNDLGWYQQKPGKAPKRLIYAASSLQSGVPSRFSGSGSGTEFTLTISSLQPEDFATYYCLQHNSYPYTFGQGTKLEIK

SEQ ID NO: 243 - DNA, 18 bp, Artificial Sequence
  synthetic
cagggcattagaaatgat

SEQ ID NO: 244 - protein, 6 aa, Artificial Sequence
  synthetic
QGIRND

SEQ ID NO: 245 - DNA, 9 bp, Artificial Sequence
  synthetic
gctgcatcc

SEQ ID NO: 246 - protein, 3 aa, Artificial Sequence
  synthetic
AAS

SEQ ID NO: 247 - DNA, 27 bp, Artificial Sequence
  synthetic
ctacagcataatagttacccgtacact

SEQ ID NO: 248 - protein, 9 aa, Artificial Sequence
  synthetic
LQHNSYPYT

SEQ ID NO: 249 - DNA, 369 bp, Artificial Sequence
  synthetic
gaagtgcagctggtggagtctgggggaggcttggttcagcctggcaggtccctgagactctcctgtgcagcctctggattcacctttgatgattttgccatgcactgggtccgacaagctccagggaagggcctggagtgggtctcaggtattagttggactggtggtaacatggactatgcgaactctgtgaagggccgattcaccatctccagagaggacgccaagaattccctgtatctgcaaatgaacagtctgagagctgcggacacggccttgtattactgtgtaaaagatataagggggatagtggctacggggggggcttttgatatctggggccgagggacaatggtcaccgtctcttca

SEQ ID NO: 250 - protein, 123 aa, Artificial Sequence
  synthetic
EVQLVESGGGLVQPGRSLRLSCAASGFTFDDFAMHWVRQAPGKGLEWVSGISWTGGNMDYANSVKGRFTISREDAKNSLYLQMNSLRAADTALYYCVKDIRGIVATGGAFDIWGRGTMVTVSS

SEQ ID NO: 251 - DNA, 24 bp, Artificial Sequence
  synthetic
ggattcacctttgatgattttgcc

SEQ ID NO: 252 - protein, 8 aa, Artificial Sequence
  synthetic
GFTFDDFA

SEQ ID NO: 253 - DNA, 24 bp, Artificial Sequence
  synthetic
attagttggactggtggtaacatg

SEQ ID NO: 254 - protein, 8 aa, Artificial Sequence
  synthetic
ISWTGGNM

SEQ ID NO: 255 - DNA, 48 bp, Artificial Sequence
  synthetic
gtaaaagatataagggggatagtggctacggggggggcttttgatatc

SEQ ID NO: 256 - protein, 16 aa, Artificial Sequence
  synthetic
VKDIRGIVATGGAFDI

SEQ ID NO: 257 - DNA, 321 bp, Artificial Sequence
  synthetic
gacatccagatgacccagtctccatcctccctgtctgcatctgtaggagacagagtcaccatctcttgccgggcaagtcagaccattagcacttatttaaattggtttcagcagaaaccagggaaagcccctaagctcctgatctatgttgtgtccagtttgcaaagtggggtcccatcaaggttcagtggcagtggatctgggacagatttcactctcaccatcagcagtctgcaacctgaagattttgcaacttattactgtcaacagagttacagtaccccattcactttcggccctgggaccaaagtggatatcaaa

SEQ ID NO: 258 - protein, 107 aa, Artificial Sequence
  synthetic
DIQMTQSPSSLSASVGDRVTISCRASQTISTYLNWFQQKPGKAPKLLIYVVSSLQSGVPSRFSGSGSGTDFTLTISSLQPEDFATYYCQQSYSTPFTFGPGTKVDIK

SEQ ID NO: 259 - DNA, 18 bp, Artificial Sequence
  synthetic
cagaccattagcacttat

SEQ ID NO: 260 - protein, 6 aa, Artificial Sequence
  synthetic
QTISTY

SEQ ID NO: 261 - DNA, 9 bp, Artificial Sequence
  synthetic
gttgtgtcc

SEQ ID NO: 262 - protein, 3 aa, Artificial Sequence
  synthetic
VVS

SEQ ID NO: 263 - DNA, 27 bp, Artificial Sequence
  synthetic
caacagagttacagtaccccattcact

SEQ ID NO: 264 - protein, 9 aa, Artificial Sequence
  synthetic
QQSYSTPFT

SEQ ID NO: 265 - DNA, 345 bp, Artificial Sequence
  synthetic
gaggtgcagctggtggagtctggaggaggcttggtccagccgggggggtccctgagactctcctgtgcagcctctggattcaccgtcggtaccaactacatgaactgggtccgccaggctccagggaagggactggagtggatctcagttatttatagcggtggtagcacattctacgcagactccgtgaagggccgattcaccatctccagacagacttcccagaacacgctgtatcttcaaatgaacagcctgagacctgaggacacggccgtatattactgtgcgagaggtatacgtggttttgatatctggggccaagggacaatggtcaccgtctcttca

SEQ ID NO: 266 - protein, 115 aa, Artificial Sequence
  synthetic
EVQLVESGGGLVQPGGSLRLSCAASGFTVGTNYMNWVRQAPGKGLEWISVIYSGGSTFYADSVKGRFTISRQTSQNTLYLQMNSLRPEDTAVYYCARGIRGFDIWGQGTMVTVSS

SEQ ID NO: 267 - DNA, 24 bp, Artificial Sequence
  synthetic
ggattcaccgtcggtaccaactac

SEQ ID NO: 268 - protein, 8 aa, Artificial Sequence
  synthetic
GFTVGTNY

SEQ ID NO: 269 - DNA, 21 bp, Artificial Sequence
  synthetic
atttatagcggtggtagcaca

SEQ ID NO: 270 - protein, 7 aa, Artificial Sequence
  synthetic
IYSGGST

SEQ ID NO: 271 - DNA, 27 bp, Artificial Sequence
  synthetic
gcgagaggtatacgtggttttgatatc

SEQ ID NO: 272 - protein, 9 aa, Artificial Sequence
  synthetic
ARGIRGFDI

SEQ ID NO: 273 - DNA, 324 bp, Artificial Sequence
  synthetic
gacatccagatgacccagtctccatcctccctgtctgcatctgtaggagacagagtcaccatcacttgccgggcaagtcagagcattagcagctatttaaattggtatcagcagaaaccagggaaagcccctaagctcctgatctatgctgcatccagtttgcaaagtggggtcccgtcaaggttcagtggcagtggatctgggacagatttcactctcaccatcagcagtctgcaacctgaagattttgcaacttactactgtcaacagagttacagtacccctccgatcaccttcggccaagggacacgactggagattaaa

SEQ ID NO: 274 - protein, 108 aa, Artificial Sequence; identical to SEQ ID NO: 194
  synthetic

SEQ ID NO: 275 - DNA, 18 bp, Artificial Sequence
  synthetic
cagagcattagcagctat

SEQ ID NO: 276 - protein, 6 aa, Artificial Sequence
  synthetic
QSISSY

SEQ ID NO: 277 - DNA, 9 bp, Artificial Sequence
  synthetic
gctgcatcc

SEQ ID NO: 278 - protein, 3 aa, Artificial Sequence
  synthetic
AAS

SEQ ID NO: 279 - DNA, 30 bp, Artificial Sequence; identical to SEQ ID NO: 95
  synthetic

SEQ ID NO: 280 - protein, 10 aa, Artificial Sequence
  synthetic
QQSYSTPPIT

SEQ ID NO: 281 - DNA, 345 bp, Artificial Sequence
  synthetic
gaggtgcagctggtggagtctggaggaggcttggtccagccgggggggtccctgagactctcctgtgcagcctctgggtttaccatcagtaccaactacatgaactgggtccgccaggctccagggaaggggctggagtgggtcgcagttatttatagcagtggttccacatactatatcgactccgtgaagggccgattcaccatctccagactcacttccaagaacacggtgtatcttcaaatgagcagcctgaattctgaagacacggccgtgtattactgtgcgagggggatcaggggttttgatatttggggccaagggacaatggtcaccgtctcttca

SEQ ID NO: 282 - protein, 115 aa, Artificial Sequence
  synthetic
EVQLVESGGGLVQPGGSLRLSCAASGFTISTNYMNWVRQAPGKGLEWVAVIYSSGSTYYIDSVKGRFTISRLTSKNTVYLQMSSLNSEDTAVYYCARGIRGFDIWGQGTMVTVSS

SEQ ID NO: 283 - DNA, 24 bp, Artificial Sequence
  synthetic
gggtttaccatcagtaccaactac

SEQ ID NO: 284 - protein, 8 aa, Artificial Sequence
  synthetic
GFTISTNY

SEQ ID NO: 285 - DNA, 21 bp, Artificial Sequence
  synthetic
atttatagcagtggttccaca

SEQ ID NO: 286 - protein, 7 aa, Artificial Sequence
  synthetic
IYSSGST

SEQ ID NO: 287 - DNA, 27 bp, Artificial Sequence
  synthetic
gcgagggggatcaggggttttgatatt

SEQ ID NO: 288 - protein, 9 aa, Artificial Sequence
  synthetic
ARGIRGFDI

SEQ ID NO: 289 - DNA, 372 bp, Artificial Sequence
  synthetic
gaagtgcagctggtggagtcggggggaggcttggtacagcctggcaggtccctgagactctcctgtgcagcctctggattcaccattgatgatagtgccatgcactgggtccggcaaactccagggaagggcctggagtgggtctcaggtattagttggaaaagtggtagcataggttatgcggactctgtgaggggccgattcaccatctccagagacaacgccaagaattccctctatctgcaaatgaacagtctgagagttgaggacacggccttgtattactgtgtaaaagatataaggggcaactggaactacgggggaaactggttcgacccctggggccagggaaccctggtcactgtctcctca

SEQ ID NO: 290 - protein, 124 aa, Artificial Sequence
  synthetic
EVQLVESGGGLVQPGRSLRLSCAASGFTIDDSAMHWVRQTPGKGLEWVSGISWKSGSIGYADSVRGRFTISRDNAKNSLYLQMNSLRVEDTALYYCVKDIRGNWNYGGNWFDPWGQGTLVTVSS

SEQ ID NO: 291 - DNA, 24 bp, Artificial Sequence
  synthetic
ggattcaccattgatgatagtgcc

SEQ ID NO: 292 - protein, 8 aa, Artificial Sequence
  synthetic
GFTIDDSA

SEQ ID NO: 293 - DNA, 24 bp, Artificial Sequence
  synthetic
attagttggaaaagtggtagcata

SEQ ID NO: 294 - protein, 8 aa, Artificial Sequence
  synthetic
ISWKSGSI

SEQ ID NO: 295 - DNA, 51 bp, Artificial Sequence
  synthetic
gtaaaagatataaggggcaactggaactacgggggaaactggttcgacccc

SEQ ID NO: 296 - protein, 17 aa, Artificial Sequence
  synthetic
VKDIRGNWNYGGNWFDP

SEQ ID NO: 297 - DNA, 345 bp, Artificial Sequence
  synthetic
gaggtgcagctggtggagtctggaggaggcttggtccagcctggggggtccctgagactctcatgtgaagcctctgggttcaccgtcggtgtcaaccacatgaactgggtccgccaggctccagggaagggtctggagtgggtctcagttattttcagtagtggtaggacattctacggagactacgtgaaggggcgattaaccatcttcagacaaacctcccagaacacggtgtatcttcaaatgaatagcctgagaagtgaggacacggccatatattactgtgcgagagggattggcggtttggacatctggggccgagggacaatggtcaccgtctcttca

SEQ ID NO: 298 - protein, 115 aa, Artificial Sequence
  synthetic
EVQLVESGGGLVQPGGSLRLSCEASGFTVGVNHMNWVRQAPGKGLEWVSVIFSSGRTFYGDYVKGRLTIFRQTSQNTVYLQMNSLRSEDTAIYYCARGIGGLDIWGRGTMVTVSS

SEQ ID NO: 299 - DNA, 24 bp, Artificial Sequence
  synthetic
gggttcaccgtcggtgtcaaccac

SEQ ID NO: 300 - protein, 8 aa, Artificial Sequence
  synthetic
GFTVGVNH

SEQ ID NO: 301 - DNA, 21 bp, Artificial Sequence
  synthetic
attttcagtagtggtaggaca

SEQ ID NO: 302 - protein, 7 aa, Artificial Sequence
  synthetic
IFSSGRT

SEQ ID NO: 303 - DNA, 27 bp, Artificial Sequence
  synthetic
gcgagagggattggcggtttggacatc

SEQ ID NO: 304 - protein, 9 aa, Artificial Sequence
  synthetic
ARGIGGLDI

SEQ ID NO: 305 - DNA, 369 bp, Artificial Sequence
  synthetic
gaagtgcagctggtggagtctgggggaggcttggttcagcctggcaggtccctaagactctcctgtgcagcctctggattcacctttgatgattatgccttgcactgggtccggcaagctccagggaagggcctggagtgggtctcaggtattagttggactggtggtactatagactatgcggactctgtgaagggccgattcaccatctccagagacaacgccaagaactccctgtatctgcaaatgagcagtctgagaactgaggacacggccatatattactgtacaagagatatccgggggaactggaagtacggaggctggttcgacccctggggccagggaaccctggtcaccgtctcctca

SEQ ID NO: 306 - protein, 123 aa, Artificial Sequence
  synthetic
EVQLVESGGGLVQPGRSLRLSCAASGFTFDDYALHWVRQAPGKGLEWVSGISWTGGTIDYADSVKGRFTISRDNAKNSLYLQMSSLRTEDTAIYYCTRDIRGNWKYGGWFDPWGQGTLVTVSS

SEQ ID NO: 307 - DNA, 24 bp, Artificial Sequence
  synthetic
ggattcacctttgatgattatgcc

SEQ ID NO: 308 - protein, 8 aa, Artificial Sequence
  synthetic
GFTFDDYA

SEQ ID NO: 309 - DNA, 24 bp, Artificial Sequence
  synthetic
attagttggactggtggtactata

SEQ ID NO: 310 - protein, 8 aa, Artificial Sequence
  synthetic
ISWTGGTI

SEQ ID NO: 311 - DNA, 48 bp, Artificial Sequence
  synthetic
acaagagatatccgggggaactggaagtacggaggctggttcgacccc

SEQ ID NO: 312 - protein, 16 aa, Artificial Sequence
  synthetic
TRDIRGNWKYGGWFDP

SEQ ID NO: 313 - DNA, 360 bp, Artificial Sequence
  synthetic
caggtgcagctggtgcagtctgggactgaggtgaagaagcctggggcctcagtgaaggtctcctgcaaggcttctggatacaccttcaccgcctactatatgcactgggtgcgacaggcccctggtcaaggacttgactggatgggatggatcagccctaacagtggtttcacaaactatgcacagaagtttcagggcagggtcaccatgaccagggacacgtccatcaacacattttatatggagctgagtggactgagatctgacgacacggccgtatattactgtgcgcgagagggttctactcaccacaattctttcgacccctggggccagggaaccctggtcaccgtctcctca

SEQ ID NO: 314 - protein, 120 aa, Artificial Sequence
  synthetic
QVQLVQSGTEVKKPGASVKVSCKASGYTFTAYYMHWVRQAPGQGLDWMGWISPNSGFTNYAQKFQGRVTMTRDTSINTFYMELSGLRSDDTAVYYCAREGSTHHNSFDPWGQGTLVTVSS

SEQ ID NO: 315 - DNA, 24 bp, Artificial Sequence
  synthetic
ggatacaccttcaccgcctactat

SEQ ID NO: 316 - protein, 8 aa, Artificial Sequence
  synthetic
GYTFTAYY

SEQ ID NO: 317 - DNA, 24 bp, Artificial Sequence
  synthetic
atcagccctaacagtggtttcaca

SEQ ID NO: 318 - protein, 8 aa, Artificial Sequence
  synthetic
ISPNSGFT

SEQ ID NO: 319 - DNA, 39 bp, Artificial Sequence
  synthetic
gcgcgagagggttctactcaccacaattctttcgacccc

SEQ ID NO: 320 - protein, 13 aa, Artificial Sequence
  synthetic
AREGSTHHNSFDP

SEQ ID NO: 321 - DNA, 342 bp, Artificial Sequence
  synthetic
gaggtgcagctggtggagtctggaggaggcttggtccaaccgggggggtccctgaggctctcctgtgcagcctctgggttcaccgtcggtactaacttcatgaattgggtccgccaggctccagggaaggggctggagtgggtctcagcgatttatagcggtggtaccgctaactacgcagactccgtgaagggccgattcaccatttccagagacacttccaggaacacgctgtatcttcaaatgaacagcctgagaactgaggacacggccgtttattattgtgcgagaggggggggtatggacgtctggggccaagggaccacggtcaccgtctcctca

SEQ ID NO: 322 - protein, 114 aa, Artificial Sequence
  synthetic
EVQLVESGGGLVQPGGSLRLSCAASGFTVGTNFMNWVRQAPGKGLEWVSAIYSGGTANYADSVKGRFTISRDTSRNTLYLQMNSLRTEDTAVYYCARGGGMDVWGQGTTVTVSS

SEQ ID NO: 323 - DNA, 24 bp, Artificial Sequence
  synthetic
gggttcaccgtcggtactaacttc

SEQ ID NO: 324 - protein, 8 aa, Artificial Sequence
  synthetic
GFTVGTNF

SEQ ID NO: 325 - DNA, 21 bp, Artificial Sequence
  synthetic
atttatagcggtggtaccgct

SEQ ID NO: 326 - protein, 7 aa, Artificial Sequence
  synthetic
IYSGGTA

SEQ ID NO: 327 - DNA, 24 bp, Artificial Sequence
  synthetic
gcgagaggggggggtatggacgtc

SEQ ID NO: 328 - protein, 8 aa, Artificial Sequence
  synthetic
ARGGGMDV

SEQ ID NO: 329 - DNA, 354 bp, Artificial Sequence
  synthetic
caggtccagctggtgcagtctggggctgaggtgaagaagcctgggtcctcggtgaaggtctcctgcaaggcttctggaggcaccttcaacacctatgttctcagctgggtgcgacaggcccctggacaagggcttgagtggatgggagagatcatccctatcttaggtgcagcaaactacgcacagaacttccagggcagagtcacttttaccacggacgaatccacgaatacagcctacatggacctgagcagcctaagatctgaggacacggccgtgtattactgtgcgagagatcggacctccggggggttcgacccctggggccagggaaccctggtcactgtctcctca

SEQ ID NO: 330 - protein, 118 aa, Artificial Sequence
  synthetic
QVQLVQSGAEVKKPGSSVKVSCKASGGTFNTYVLSWVRQAPGQGLEWMGEIIPILGAANYAQNFQGRVTFTTDESTNTAYMDLSSLRSEDTAVYYCARDRTSGGFDPWGQGTLVTVSS

SEQ ID NO: 331 - DNA, 24 bp, Artificial Sequence
  synthetic
ggaggcaccttcaacacctatgtt

SEQ ID NO: 332 - protein, 8 aa, Artificial Sequence
  synthetic
GGTFNTYV

SEQ ID NO: 333 - DNA, 24 bp, Artificial Sequence
  synthetic
atcatccctatcttaggtgcagca

SEQ ID NO: 334 - protein, 8 aa, Artificial Sequence
  synthetic
IIPILGAA

SEQ ID NO: 335 - DNA, 33 bp, Artificial Sequence
  synthetic
gcgagagatcggacctccggggggttcgacccc

SEQ ID NO: 336 - protein, 11 aa, Artificial Sequence
  synthetic
ARDRTSGGFDP

SEQ ID NO: 337 - DNA, 357 bp, Artificial Sequence
  synthetic
caggttcagctggtgcagtctggagctgaggtggagaagcctggggcctcagtgaaggtctcctgcaaggcttctggttacatctttacccactatggtatcagctgggtgcgacaggcccctggacaaggacttgagtgggtgggctggatcagcccttacaatggttacacagactatgcacagaaactccagggcagagtcaccttgaccacagacacatccacgaccacagcctacatggagctgaggaacctgagatctgacgacacggccatgtattactgttcgagagggaggggcccttactggtccttcgatctctggggccgtggcaccctggtcaccgtctcctca

SEQ ID NO: 338 - protein, 119 aa, Artificial Sequence
  synthetic
QVQLVQSGAEVEKPGASVKVSCKASGYIFTHYGISWVRQAPGQGLEWVGWISPYNGYTDYAQKLQGRVTLTTDTSTTTAYMELRNLRSDDTAMYYCSRGRGPYWSFDLWGRGTLVTVSS

SEQ ID NO: 339 - DNA, 24 bp, Artificial Sequence
  synthetic
ggttacatctttacccactatggt

SEQ ID NO: 340 - protein, 8 aa, Artificial Sequence
  synthetic
GYIFTHYG

SEQ ID NO: 341 - DNA, 24 bp, Artificial Sequence
  synthetic
atcagcccttacaatggttacaca

SEQ ID NO: 342 - protein, 8 aa, Artificial Sequence
  synthetic
ISPYNGYT

SEQ ID NO: 343 - DNA, 36 bp, Artificial Sequence
  synthetic
tcgagagggaggggcccttactggtccttcgatctc

SEQ ID NO: 344 - protein, 12 aa, Artificial Sequence
  synthetic
SRGRGPYWSFDL